European Patent Specification EP 3 870 698 B1, published March 18, 2026. Title: Antipathogenic Polypeptides. Applicant: University of Virginia Patent Foundation. The sequence listing filed with the application follows.

SEQUENCE LISTING (6 sequences)

SEQ ID NO: 1 - protein, 742 aa, Stenotrophomonas maltophilia
MRLQPLFVSLALAAPCALLPTASLSAAPAAAARQADTAPVLVTAAQWQQMASEGRRYPWFAKEQARTEATLKKMMKAGIDVPVPRDKGGGRTHEQHKRNYQALLAAGTLYRLTGDRAYVDYARDMLLQYAQLYPTLGPHPEGRGQIPGRVFWQVLNDSVWLVNAIQGYDAIRDALSAEDRNTIESKVFRPMAEFLVSEPKNYDQIHNHATWAVAATGMTGYVLRDQELVEKSLRGSQKDDKFGFLRQIDLLFSPDGYYEEGPYYQRYALAPFLLFANAIERNEPQRKIFARRDGVLLKAVDVLVQSSYGGLFFPINDAILDKGIDTEELVAGIGIAYARTGDDRLLSVAEQQKRLLLSPEGLQVAQALAANKAKPFDYHPMLLRDGPDGDRGGLAILRMNGERGQALVQKDTMQGMGHGHFDKLNWLFYDNGNPVVTDYGAARFLNVEAKRGGIYLAENRSWAKQTVAHNTLVVDEQSHFNGNWKRGEAHAPQVRFFQADADTQIASATMRDAYPGVAFTRTQALLRHPDLGLPVVLDLLQVHGDKAARYDLPLHFNGHIVTTGFEAEHFPSQRPVLGKDNGYQHLWLDARSKPGSEPRSLAWLLDGRFYTYRFGSSAPAQALLVESGANDPEFNLRREPALLQRVDGQKDVTFFSVLEPHGEYNGTAEYVHGADSRIREIVRTRGSDAEVIELRLASGARIALGVADNSATTSEHSVTVDGHVYRWNGSHARLDRSKGDGK

SEQ ID NO: 2 - protein, 742 aa, Artificial Sequence
  Synthesized - Modified Stenotrophomonas maltophilia (Smlt2602) (W152F)
MRLQPLFVSLALAAPCALLPTASLSAAPAAAARQADTAPVLVTAAQWQQMASEGRRYPWFAKEQARTEATLKKMMKAGIDVPVPRDKGGGRTHEQHKRNYQALLAAGTLYRLTGDRAYVDYARDMLLQYAQLYPTLGPHPEGRGQIPGRVFFQVLNDSVWLVNAIQGYDAIRDALSAEDRNTIESKVFRPMAEFLVSEPKNYDQIHNHATWAVAATGMTGYVLRDQELVEKSLRGSQKDDKFGFLRQIDLLFSPDGYYEEGPYYQRYALAPFLLFANAIERNEPQRKIFARRDGVLLKAVDVLVQSSYGGLFFPINDAILDKGIDTEELVAGIGIAYARTGDDRLLSVAEQQKRLLLSPEGLQVAQALAANKAKPFDYHPMLLRDGPDGDRGGLAILRMNGERGQALVQKDTMQGMGHGHFDKLNWLFYDNGNPVVTDYGAARFLNVEAKRGGIYLAENRSWAKQTVAHNTLVVDEQSHFNGNWKRGEAHAPQVRFFQADADTQIASATMRDAYPGVAFTRTQALLRHPDLGLPVVLDLLQVHGDKAARYDLPLHFNGHIVTTGFEAEHFPSQRPVLGKDNGYQHLWLDARSKPGSEPRSLAWLLDGRFYTYRFGSSAPAQALLVESGANDPEFNLRREPALLQRVDGQKDVTFFSVLEPHGEYNGTAEYVHGADSRIREIVRTRGSDAEVIELRLASGARIALGVADNSATTSEHSVTVDGHVYRWNGSHARLDRSKGDGK

SEQ ID NO: 3 - protein, 742 aa, Artificial Sequence
  Synthesized - Modified Stenotrophomonas maltophilia (Smlt2602) (Y202F)
MRLQPLFVSLALAAPCALLPTASLSAAPAAAARQADTAPVLVTAAQWQQMASEGRRYPWFAKEQARTEATLKKMMKAGIDVPVPRDKGGGRTHEQHKRNYQALLAAGTLYRLTGDRAYVDYARDMLLQYAQLYPTLGPHPEGRGQIPGRVFWQVLNDSVWLVNAIQGYDAIRDALSAEDRNTIESKVFRPMAEFLVSEPKNFDQIHNHATWAVAATGMTGYVLRDQELVEKSLRGSQKDDKFGFLRQIDLLFSPDGYYEEGPYYQRYALAPFLLFANAIERNEPQRKIFARRDGVLLKAVDVLVQSSYGGLFFPINDAILDKGIDTEELVAGIGIAYARTGDDRLLSVAEQQKRLLLSPEGLQVAQALAANKAKPFDYHPMLLRDGPDGDRGGLAILRMNGERGQALVQKDTMQGMGHGHFDKLNWLFYDNGNPVVTDYGAARFLNVEAKRGGIYLAENRSWAKQTVAHNTLVVDEQSHFNGNWKRGEAHAPQVRFFQADADTQIASATMRDAYPGVAFTRTQALLRHPDLGLPVVLDLLQVHGDKAARYDLPLHFNGHIVTTGFEAEHFPSQRPVLGKDNGYQHLWLDARSKPGSEPRSLAWLLDGRFYTYRFGSSAPAQALLVESGANDPEFNLRREPALLQRVDGQKDVTFFSVLEPHGEYNGTAEYVHGADSRIREIVRTRGSDAEVIELRLASGARIALGVADNSATTSEHSVTVDGHVYRWNGSHARLDRSKGDGK

SEQ ID NO: 4 - protein, 742 aa, Artificial Sequence
  Synthesized - Modified Stenotrophomonas maltophilia (Smlt2602) (Y202F, H208F)
MRLQPLFVSLALAAPCALLPTASLSAAPAAAARQADTAPVLVTAAQWQQMASEGRRYPWFAKEQARTEATLKKMMKAGIDVPVPRDKGGGRTHEQHKRNYQALLAAGTLYRLTGDRAYVDYARDMLLQYAQLYPTLGPHPEGRGQIPGRVFWQVLNDSVWLVNAIQGYDAIRDALSAEDRNTIESKVFRPMAEFLVSEPKNFDQIHNFATWAVAATGMTGYVLRDQELVEKSLRGSQKDDKFGFLRQIDLLFSPDGYYEEGPYYQRYALAPFLLFANAIERNEPQRKIFARRDGVLLKAVDVLVQSSYGGLFFPINDAILDKGIDTEELVAGIGIAYARTGDDRLLSVAEQQKRLLLSPEGLQVAQALAANKAKPFDYHPMLLRDGPDGDRGGLAILRMNGERGQALVQKDTMQGMGHGHFDKLNWLFYDNGNPVVTDYGAARFLNVEAKRGGIYLAENRSWAKQTVAHNTLVVDEQSHFNGNWKRGEAHAPQVRFFQADADTQIASATMRDAYPGVAFTRTQALLRHPDLGLPVVLDLLQVHGDKAARYDLPLHFNGHIVTTGFEAEHFPSQRPVLGKDNGYQHLWLDARSKPGSEPRSLAWLLDGRFYTYRFGSSAPAQALLVESGANDPEFNLRREPALLQRVDGQKDVTFFSVLEPHGEYNGTAEYVHGADSRIREIVRTRGSDAEVIELRLASGARIALGVADNSATTSEHSVTVDGHVYRWNGSHARLDRSKGDGK

SEQ ID NO: 5 - protein, 742 aa, Artificial Sequence
  Synthesized - Modified Stenotrophomonas maltophilia (Smlt2602) (Q153A)
MRLQPLFVSLALAAPCALLPTASLSAAPAAAARQADTAPVLVTAAQWQQMASEGRRYPWFAKEQARTEATLKKMMKAGIDVPVPRDKGGGRTHEQHKRNYQALLAAGTLYRLTGDRAYVDYARDMLLQYAQLYPTLGPHPEGRGQIPGRVFWAVLNDSVWLVNAIQGYDAIRDALSAEDRNTIESKVFRPMAEFLVSEPKNYDQIHNHATWAVAATGMTGYVLRDQELVEKSLRGSQKDDKFGFLRQIDLLFSPDGYYEEGPYYQRYALAPFLLFANAIERNEPQRKIFARRDGVLLKAVDVLVQSSYGGLFFPINDAILDKGIDTEELVAGIGIAYARTGDDRLLSVAEQQKRLLLSPEGLQVAQALAANKAKPFDYHPMLLRDGPDGDRGGLAILRMNGERGQALVQKDTMQGMGHGHFDKLNWLFYDNGNPVVTDYGAARFLNVEAKRGGIYLAENRSWAKQTVAHNTLVVDEQSHFNGNWKRGEAHAPQVRFFQADADTQIASATMRDAYPGVAFTRTQALLRHPDLGLPVVLDLLQVHGDKAARYDLPLHFNGHIVTTGFEAEHFPSQRPVLGKDNGYQHLWLDARSKPGSEPRSLAWLLDGRFYTYRFGSSAPAQALLVESGANDPEFNLRREPALLQRVDGQKDVTFFSVLEPHGEYNGTAEYVHGADSRIREIVRTRGSDAEVIELRLASGARIALGVADNSATTSEHSVTVDGHVYRWNGSHARLDRSKGDGK

SEQ ID NO: 6 - protein, 742 aa, Artificial Sequence
  Synthesized - Modified Stenotrophomonas maltophilia (Smlt2602) (Y455F)
MRLQPLFVSLALAAPCALLPTASLSAAPAAAARQADTAPVLVTAAQWQQMASEGRRYPWFAKEQARTEATLKKMMKAGIDVPVPRDKGGGRTHEQHKRNYQALLAAGTLYRLTGDRAYVDYARDMLLQYAQLYPTLGPHPEGRGQIPGRVFWQVLNDSVWLVNAIQGYDAIRDALSAEDRNTIESKVFRPMAEFLVSEPKNYDQIHNHATWAVAATGMTGYVLRDQELVEKSLRGSQKDDKFGFLRQIDLLFSPDGYYEEGPYYQRYALAPFLLFANAIERNEPQRKIFARRDGVLLKAVDVLVQSSYGGLFFPINDAILDKGIDTEELVAGIGIAYARTGDDRLLSVAEQQKRLLLSPEGLQVAQALAANKAKPFDYHPMLLRDGPDGDRGGLAILRMNGERGQALVQKDTMQGMGHGHFDKLNWLFYDNGNPVVTDYGAARFLNVEAKRGGIFLAENRSWAKQTVAHNTLVVDEQSHFNGNWKRGEAHAPQVRFFQADADTQIASATMRDAYPGVAFTRTQALLRHPDLGLPVVLDLLQVHGDKAARYDLPLHFNGHIVTTGFEAEHFPSQRPVLGKDNGYQHLWLDARSKPGSEPRSLAWLLDGRFYTYRFGSSAPAQALLVESGANDPEFNLRREPALLQRVDGQKDVTFFSVLEPHGEYNGTAEYVHGADSRIREIVRTRGSDAEVIELRLASGARIALGVADNSATTSEHSVTVDGHVYRWNGSHARLDRSKGDGK